European Patent Application EP 4 644 572 A1, published November 5, 2025. Title: Method for analysing trait purity in large seed bulks. Applicant: KWS SAAT SE & CO KGaA. The sequence listing filed with the application follows.

SEQUENCE LISTING (6 sequences)

SEQ ID NO: 1 - DNA, 21 bp, synthetic construct
  source 1..21: mol_type = other DNA
tgatgcaaataggctgggaat

SEQ ID NO: 2 - DNA, 22 bp, synthetic construct
  source 1..22: mol_type = other DNA
agcgcgcaaactaggataaatt

SEQ ID NO: 3 - DNA, 22 bp, synthetic construct
  source 1..22: mol_type = other DNA
tgccttatctgttgccttcaga

SEQ ID NO: 4 - DNA, 24 bp, synthetic construct
  source 1..24: mol_type = other DNA
gccagtaaaacaactacccatggt

SEQ ID NO: 5 - DNA, 20 bp, synthetic construct
  source 1..20: mol_type = other DNA
gagcgcatcgtcactgctga

SEQ ID NO: 6 - DNA, 20 bp, synthetic construct
  source 1..20: mol_type = other DNA
gcgcgcggtgtcatctatgt